European Patent Application EP 4 438 719 A1, published October 2, 2024. Title: 工程化迁移体及其制备方法和用途. Applicant: 北京迈格松生物科技有限公司. The sequence listing filed with the application follows.

SEQUENCE LISTING (7 sequences)

SEQ ID NO: 1 - protein, 479 aa, synthetic construct
  REGION 1..479: note = Tspan4-linker-GFP
MARGCLQGVKYLMFAFNLLFWLGGCGVLGVGIWLAATQGNFATLSSSFPSLSAANLLIVTGTFVMAIGFVGCIGALKENKCLLLTFFVLLLLVFLLEATIAVLFFAYSDKIDSYAQQDLKKGLHLYGTQGNVGLTNAWSIIQTDFRCCGVSNYTDWFEVYNATRVPDSCCLEFSDSCGLHEPGTWWKSPCYETVKAWLQENLLAVGIFGLCTALVQILGLTFAMTMYCQVVKADTYCAPGMVSKGEELFTGVVPILVELDGDVNGHKFSVSGEGEGDATYGKLTLKFICTTGKLPVPWPTLVTTLTYGVQCFSRYPDHMKQHDFFKSAMPEGYVQERTIFFKDDGNYKTRAEVKFEGDTLVNRIELKGIDFKEDGNILGHKLEYNYNSHNVYIMADKQKNGIKVNFKIRHNIEDGSVQLADHYQQNTPIGDGPVLLPDNHYLSTQSALSKDPNEKRDHMVLLEFVTAAGITLGMDELYK

SEQ ID NO: 2 - protein, 1136 aa, synthetic construct
  REGION 1..1136: note = DAG1-linker-mCherry
MSVDNWLLHPLWGQTFLLLLSVAVAQAHWPSEPSEAVRDWKNQLEASMHSVLSDFQEAVPTVVGIPDGTAVVGRSFRVSIPTDLIASSGEIIKVSAAGKEALPSWLHWDPHSHILEGLPLDTDKGVHYISVSAARLGANGSHVPQTASVFSIEVYPEDHSEPQSVRAASSDPGEVVSSACAADEPVTVLTVILDADLTKMTPKQRIDLLNRMQSFSEVELNNMKLVPVVNNRLFDMSAFMAGPGNAKKVVENGALLSWKLGCSLNQNSVPDIRGVETPAREGTMSAHLGYPVVGWHIANKKPTLPKRIRRQIHATPTPVTAIGPPTTAIQEPPSRIVPTPTSPAIAPPTETMAPPVRDPVPGKPTVTIRTRGAIIQTPTLGPIPPTRVSEAGTTVPGQIRPTLTIPGYVEPTAVVTPPTTTTKKPRVSTPKPATPSTDSSTTTTRRPTKKPRTPRPVPRVTTKAPITRLETASPPTRIRTTTSAVPRGGEANQRPELKNHIDRVDAWVGTYFEVKIPSDTFYDNEDTTTDKLKLTLKLREQQLVGEKSWVQFNSNSQLMYGLPDSSHVGKHEYFMHATDKGGLSAVDAFEIHVHKRPQGDKAPARFKAKLAGDPAPVVNDIHKKIALVKKLAFAFGDRNCSSITLQNITRGSIVVEWTNNTLPLEPCPKEQIVGLSRRIADENGKPRPAFSNALEPDFKALSVAVAGSGSCRHLQFIPVAPPSPGTSAAPATEVPDRDPEKSSEDDVYLHTVIPAVVVAAILLIAGIIAMICYRKKRKGKLTLEDQATFIKKGVPIIFADELDDSKPPPSSSMPLILQEEKAPLPPPEYPNQSVPETTPLNQDTVGEYTPLRDEDPNAPPYQPPPPFTAPMEGKGSRPKNMTPYRSPPPYVPPGDPPVATMVSKGEEDNMAIIKEFMRFKVHMEGSVNGHEFEIEGEGEGRPYEGTQTAKLKVTKGGPLPFAWDILSPQFMYGSKAYVKHPADIPDYLKLSFPEGFKWERVMNFEDGGVVTVTQDSSLQDGEFIYKVKLRGTNFPSDGPVMQKKTMGWEASSERMYPEDGALKGEIKQRLKLKDGGHYDAEVKTTYKAKKPVQLPGAYNVNIKLDITSHNEDYTIVEQYERAEGRHSTGGMDELYK

SEQ ID NO: 3 - protein, 536 aa, synthetic construct
  REGION 1..536: note = PDCD1-linker-mCherry
MWVRQVPWSFTWAVLQLSWQSGWLLEVPNGPWRSLTFYPAWLTVSEGANATFTCSLSNWSEDLMLNWNRLSPSNQTEKQAAFCNGLSQPVQDARFQIIQLPNRHDFHMNILDTRRNDSGIYLCGAISLHPKAKIEESPGAELVVTERILETSTRYPSPSPKPEGRFQGMVIGIMSALVGIPVLLLLAWALAVFCSTSMSEARGAGSKDDTLKEEPSAAPVPSVAYEELDFQGREKTPELPTACVHTEYATIVFTEGLGASAMGRRGSADGLQGPRPPRHEDGHCSWPLTVPRARDPPVATMVSKGEEDNMAIIKEFMRFKVHMEGSVNGHEFEIEGEGEGRPYEGTQTAKLKVTKGGPLPFAWDILSPQFMYGSKAYVKHPADIPDYLKLSFPEGFKWERVMNFEDGGVVTVTQDSSLQDGEFIYKVKLRGTNFPSDGPVMQKKTMGWEASSERMYPEDGALKGEIKQRLKLKDGGHYDAEVKTTYKAKKPVQLPGAYNVNIKLDITSHNEDYTIVEQYERAEGRHSTGGMDELYK

SEQ ID NO: 4 - protein, 751 aa, synthetic construct
  REGION 1..751: note = Tgfbr1-linker-mCherry
MEAAAAAPRRPQLLIVLVAAATLLPGAKALQCFCHLCTKDNFTCETDGLCFVSVTETTDKVIHNSMCIAEIDLIPRDRPFVCAPSSKTGAVTTTYCCNQDHCNKIELPTTGPFSEKQSAGLGPVELAAVIAGPVCFVCIALMLMVYICHNRTVIHHRVPNEEDPSLDRPFISEGTTLKDLIYDMTTSGSGSGLPLLVQRTIARTIVLQESIGKGRFGEVWRGKWRGEEVAVKIFSSREERSWFREAEIYQTVMLRHENILGFIAADNKDNGTWTQLWLVSDYHEHGSLFDYLNRYTVTVEGMIKLALSTASGLAHLHMEIVGTQGKPAIAHRDLKSKNILVKKNGTCCIADLGLAVRHDSATDTIDIAPNHRVGTKRYMAPEVLDDSINMKHFESFKRADIYAMGLVFWEIARRCSIGGIHEDYQLPYYDLVPSDPSVEEMRKVVCEQKLRPNIPNRWQSCEALRVMAKIMRECWYANGAARLTALRIKKTLSQLSQQEGIKMTVPRARDPPVATMVSKGEEDNMAIIKEFMRFKVHMEGSVNGHEFEIEGEGEGRPYEGTQTAKLKVTKGGPLPFAWDILSPQFMYGSKAYVKHPADIPDYLKLSFPEGFKWERVMNFEDGGVVTVTQDSSLQDGEFIYKVKLRGTNFPSDGPVMQKKTMGWEASSERMYPEDGALKGEIKQRLKLKDGGHYDAEVKTTYKAKKPVQLPGAYNVNIKLDITSHNEDYTIVEQYERAEGRHSTGGMDELYK

SEQ ID NO: 5 - protein, 431 aa, synthetic construct
  REGION 1..431: note = mCherry-linker-Kras
MVSKGEEDNMAIIKEFMRFKVHMEGSVNGHEFEIEGEGEGRPYEGTQTAKLKVTKGGPLPFAWDILSPQFMYGSKAYVKHPADIPDYLKLSFPEGFKWERVMNFEDGGVVTVTQDSSLQDGEFIYKVKLRGTNFPSDGPVMQKKTMGWEASSERMYPEDGALKGEIKQRLKLKDGGHYDAEVKTTYKAKKPVQLPGAYNVNIKLDITSHNEDYTIVEQYERAEGRHSTGGMDELYKSGLRSRGMTEYKLVVVGAGGVGKSALTIQLIQNHFVDEYDPTIEDSYRKQVVIDGETCLLDILDTAGQEEYSAMRDQYMRTGEGFLCVFAINNTKSFEDIHHYREQIKRVKDSEDVPMVLVGNKCDLPSRTVDTKQAQELARSYGIPFIETSAKTRQGVDDAFYTLVREIRKHKEKMSKDGKKKKKKSRTRCIVM

SEQ ID NO: 6 - protein, 670 aa, synthetic construct
  REGION 1..670: note = t-STX2-linker-OVA-linker-mCherry
MKKAIKYQSKARRKKWIIAAVAVAVIAVLALIIGLSVGKGSMGSIGAASMEFCFDVFKELKVHHANENIFYCPIAIMSALAMVYLGAKDSTRTQINKVVRFDKLPGFGDSIEAQCGTSVNVHSSLRDILNQITKPNDVYSFSLASRLYAEERYPILPEYLQCVKELYRGGLEPINFQTAADQARELINSWVESQTNGIIRNVLQPSSVDSQTAMVLVNAIVFKGLWEKAFKDEDTQAMPFRVTEQESKPVQMMYQIGLFRVASMASEKMKILELPFASGTMSMLVLLPDEVSGLEQLESIINFEKLTEWTSSNVMEERKIKVYLPRMKMEEKYNLTSVLMAMGITDVFSSSANLSGISSAESLKISQAVHAAHAEINEAGREVVGSAEAGVDAASVSEEFRADHPFLFCIKHIATNAVLFFGRCVSPGDPPVATMVSKGEEDNMAIIKEFMRFKVHMEGSVNGHEFEIEGEGEGRPYEGTQTAKLKVTKGGPLPFAWDILSPQFMYGSKAYVKHPADIPDYLKLSFPEGFKWERVMNFEDGGVVTVTQDSSLQDGEFIYKVKLRGTNFPSDGPVMQKKTMGWEASSERMYPEDGALKGEIKQRLKLKDGGHYDAEVKTTYKAKKPVQLPGAYNVNIKLDITSHNEDYTIVEQYERAEGRHSTGGMDELYK

SEQ ID NO: 7 - protein, 778 aa, synthetic construct
  REGION 1..778: note = Tspan4-linker-GFP-linker-Halo
MARGCLQGVKYLMFAFNLLFWLGGCGVLGVGIWLAATQGNFATLSSSFPSLSAANLLIVTGTFVMAIGFVGCIGALKENKCLLLTFFVLLLLVFLLEATIAVLFFAYSDKIDSYAQQDLKKGLHLYGTQGNVGLTNAWSIIQTDFRCCGVSNYTDWFEVYNATRVPDSCCLEFSDSCGLHEPGTWWKSPCYETVKAWLQENLLAVGIFGLCTALVQILGLTFAMTMYCQVVKADTYCAPGMVSKGEELFTGVVPILVELDGDVNGHKFSVSGEGEGDATYGKLTLKFICTTGKLPVPWPTLVTTLTYGVQCFSRYPDHMKQHDFFKSAMPEGYVQERTIFFKDDGNYKTRAEVKFEGDTLVNRIELKGIDFKEDGNILGHKLEYNYNSHNVYIMADKQKNGIKVNFKIRHNIEDGSVQLADHYQQNTPIGDGPVLLPDNHYLSTQSALSKDPNEKRDHMVLLEFVTAAGITLGMDELYKGSMAEIGTGFPFDPHYVEVLGERMHYVDVGPRDGTPVLFLHGNPTSSYVWRNIIPHVAPTHRCIAPDLIGMGKSDKPDLGYFFDDHVRFMDAFIEALGLEEVVLVIHDWGSALGFHWAKRNPERVKGIAFMEFIRPIPTWDEWPEFARETFQAFRTTDVGRKLIIDQNVFIEGTLPMGVVRPLTEVEMDHYREPFLNPVDREPLWRFPNELPIAGEPANIVALVEEYMDWLHQSPVPKLLFWGTPGVLIPPAEAARLAKSLPNCKAVDIGPGLNLLQEDNPDLIGSEIARWLSTLEISG